European Patent Application EP 4 335 859 A1, published March 13, 2024. Title: A method for designing oligonucleotides with reduced central toxicity. Applicant: Luxna Biotech Co., Ltd. Application 22798959.7. The sequence listing filed with the application follows.

SEQUENCE LISTING (8 sequences)

SEQ ID NO: 1 - DNA, 16 bp, Artificial Sequence
  LX-A4285
  misc_feature (1)..(1): a = LNA-a
  misc_feature (2)..(3): c = LNA-5-methylcytosine
  misc_feature (14)..(14): g = LNA-g
  misc_feature (15)..(15): c = LNA-5-methylcytosine
  misc_feature (16)..(16): t = LNA-t
accatgatcttaggct

SEQ ID NO: 2 - DNA, 16 bp, Artificial Sequence
  LX-A5105
  misc_feature (1)..(1): a = LNA-a
  misc_feature (2)..(3): c = LNA-5-methylcytosine
  misc_feature (4)..(4): a = 5'-cyclopropane-2'-deoxyadenosine (5'-cp-A)
  misc_feature (14)..(14): g = LNA-g
  misc_feature (15)..(15): c = LNA-5-methylcytosine
  misc_feature (16)..(16): t = LNA-t
accatgatcttaggct

SEQ ID NO: 3 - DNA, 16 bp, Artificial Sequence
  LX-A5106
  misc_feature (1)..(1): a = LNA-a
  misc_feature (2)..(3): c = LNA-5-methylcytosine
  misc_feature (4)..(4): a = 5'-cyclopropane-2'-deoxyadenosine (5'-cp-A)
  misc_feature (5)..(5): t = 5'-cyclopropanethymidine (5'-cp-T)
  misc_feature (14)..(14): g = LNA-g
  misc_feature (15)..(15): c = LNA-5-methylcytosine
  misc_feature (16)..(16): t = LNA-t
accatgatcttaggct

SEQ ID NO: 4 - DNA, 16 bp, Artificial Sequence
  LX-A5107
  misc_feature (1)..(1): a = LNA-a
  misc_feature (2)..(3): c = LNA-5-methylcytosine
  misc_feature (4)..(4): a = 5'-cyclopropane-2'-deoxyadenosine (5'-cp-A)
  misc_feature (5)..(5): t = 5'-cyclopropanethymidine (5'-cp-T)
  misc_feature (6)..(6): g = 5'-cyclopropane-2'-deoxyguanosine (5'-cp-G)
  misc_feature (14)..(14): g = LNA-g
  misc_feature (15)..(15): c = LNA-5-methylcytosine
  misc_feature (16)..(16): t = LNA-t
accatgatcttaggct

SEQ ID NO: 5 - DNA, 16 bp, Artificial Sequence
  LX-A5108
  misc_feature (1)..(1): a = LNA-a
  misc_feature (2)..(3): c = LNA-5-methylcytosine
  misc_feature (4)..(4): a = 5'-cyclopropane-2'-deoxyadenosine (5'-cp-A)
  misc_feature (5)..(5): t = 5'-cyclopropanethymidine (5'-cp-T)
  misc_feature (6)..(6): g = 5'-cyclopropane-2'-deoxyguanosine (5'-cp-G)
  misc_feature (7)..(7): a = 5'-cyclopropane-2'-deoxyadenosine (5'-cp-A)
  misc_feature (14)..(14): g = LNA-g
  misc_feature (15)..(15): c = LNA-5-methylcytosine
  misc_feature (16)..(16): t = LNA-t
accatgatcttaggct

SEQ ID NO: 6 - DNA, 15 bp, Artificial Sequence
  LX-A0070
  misc_feature (1)..(1): c = AmNA-5-methylcytosine
  misc_feature (2)..(2): a = AmNA-a
  misc_feature (3)..(3): t = AmNA-t
  misc_feature (13)..(13): c = AmNA-5-methylcytosine
  misc_feature (14)..(14): t = AmNA-t
catttagaagtcctc

SEQ ID NO: 7 - DNA, 16 bp, Artificial Sequence
  LX-A4286
  misc_feature (1)..(1): a = LNA-a
  misc_feature (2)..(3): c = LNA-5-methylcytosine
  misc_feature (14)..(14): g = LNA-g
  misc_feature (15)..(15): c = LNA-5-methylcytosine
  misc_feature (16)..(16): t = LNA-t
accatgatcttaggct

SEQ ID NO: 8 - DNA, 16 bp, Artificial Sequence
  LX-A5113
  misc_feature (1)..(1): a = LNA-a
  misc_feature (2)..(3): c = LNA-5-methylcytosine
  misc_feature (4)..(4): a = 5'-cyclopropane-2'-deoxyadenosine (5'-cp-A)
  misc_feature (5)..(5): t = 5'-cyclopropanethymidine (5'-cp-T)
  misc_feature (12)..(12): a = 5'-cyclopropane-2'-deoxyadenosine (5'-cp-A)
  misc_feature (13)..(13): g = 5'-cyclopropane-2'-deoxyguanosine (5'-cp-G)
  misc_feature (14)..(14): g = LNA-g
  misc_feature (15)..(15): c = LNA-5-methylcytosine
  misc_feature (16)..(16): t = LNA-t
accatgatcttaggct